European Patent Specification EP 4 070 808 B1, published September 18, 2024. Title: Pharmaceutical composition for preventing or treating Behcets disease and rheumatoid arthritis comprising peptides of snake venom or mixture thereof. Applicant: AJOU UNIVERSITY INDUSTRY-ACADEMIC COOPERATION FOUNDATION. The sequence listing filed with the application follows.

SEQUENCE LISTING (5 sequences)

SEQ ID NO: 1 - protein, 13 aa, Unknown
  3-finger toxin
LICPEKYCNKVHT

SEQ ID NO: 2 - protein, 11 aa, Unknown
  3-finger toxin
YCNKVHTCRNG

SEQ ID NO: 3 - protein, 15 aa, Unknown
  3-finger toxin
PREIVECCSTDKCNH

SEQ ID NO: 4 - protein, 11 aa, Unknown
  3-finger toxin
HTCRNGENICF

SEQ ID NO: 5 - protein, 23 aa, Unknown
  3-finger toxin
ENICFKRFYEGNLLGKRYPRGCA